European Patent Specification EP 3 876 921 B1, published August 26, 2026. Title: METHODS FOR INHIBITING CONVERSION OF CHOLINE TO TRIMETHYLAMINE (TMA). Applicant: The Procter & Gamble Company. The sequence listing filed with the application follows.

SEQUENCE LISTING (2 sequences)

SEQ ID NO: 1 - DNA, 419 bp, Mikania guaco
actttcctctttgacgtaacccaacgccctggcacaagccaatgcgagttgagcagtcgtatacgagaagcataaccaggacataaaaggaactcacgaaacccatgcccacatcagttccataccaaagataccaagcaattaccaatgtaccacatcaccagacaagcatcagagaggtggttcaaggagttgccttcatggttcatccgatctcataaagtacaagacaagacgaaagaacttataccagccaacaaaagtaccacatgataggtaggcaacacaggaaacccacaatctgttttagcaatagaagccttaacagacaaatgaaaaggtatgtcaggtggaagttgttgcacaagcaaagagccaaccaccagtaacaaaccaaacaccactcatgcacctttacg

SEQ ID NO: 2 - DNA, 714 bp, Mikania guaco
aagtcgtaacaaggtttccgtaggtgaacctgcggaaggatcattgtcgaatcctgcgtagcagaacaacctgtgaacgtgtaacaacaaaatggcttcactgggggtgttgcttttgtttcagaccctgtgaagccttttcagcacgtgtttgtggttgcctgtttcggtcactcatggatgtcgtgctgatgtaacaaccccccggcacaacatgtgccaaggaaatcaaatcttaagagggcatgtgccatgacaccccgtacgtggtgtgtttgtcgtatgtggcccctatgtaaaatcttaaaacaactctcggcaacggatatcttggctcacgcatcgatgaagaacgtagcaaaatgcgatacttggtgtgaattgcagaatcccgtgaaccatcgagtttttgaacgcaagttgcgcccgaagccacttggttgagggcacgtctgcctgggtgtcacgcatcatgtcgcccaaatcaaacttaccttagggtactgtgttgtatgtagggcggagactggtctcctatgcccatggcgtggttggccgaaatacgagtcccttgacgagtgacgcatgactggtggtggttgattagacagtcgtcctgtgtcgtgcgtttataattgtgatgggaaaaggctcttaaaataccctgatatgtgttgtctagtgacaattgtttgattgcgaccccaggtcagg